European Patent Application EP 4 644 568 A2, published November 5, 2025. Title: Methods for targeted nucleic acid library formation. Applicant: Agilent Technologies, Inc. Application EP. The sequence listing filed with the application follows.

SEQUENCE LISTING (15 sequences)

SEQ ID NO: 1 - DNA, 70 bp, synthetic construct
  misc_feature 1..70: note = Description of Artificial Sequence: Synthetic oligonucleotide
  misc_feature 70: note = n = a, c, t, or g
  source 1..70: mol_type = other DNA
cgtcgctatcaaggaattaagagaagcaacatctccgaaagccaacaaggaaatcctcgatgtgagtttn

SEQ ID NO: 2 - DNA, 50 bp, synthetic construct
  misc_feature 1..50: note = Description of Artificial Sequence: Synthetic probe
  misc_feature 2..4: note = n = a, c, t, or g
  source 1..50: mol_type = other DNA
gnnngatcgtcggactgtagaactctgaaccgaacgacgacatagaccac

SEQ ID NO: 3 - DNA, 59 bp, synthetic construct
  misc_feature 1..59: note = Description of Artificial Sequence: Synthetic probe
  source 1..59: mol_type = other DNA
gtggtctatgtcgtcgttcgtttttttttttttttcttgttggctttcggagatgttgc

SEQ ID NO: 4 - DNA, 26 bp, synthetic construct
  misc_feature 1..26: note = Description of Artificial Sequence: Synthetic primer
  source 1..26: mol_type = other DNA
gttcagagttctacagtccgacgatc

SEQ ID NO: 5 - DNA, 21 bp, synthetic construct
  misc_feature 1..21: note = Description of Artificial Sequence: Synthetic primer
  source 1..21: mol_type = other DNA
cgtcgctatcaaggaattaag

SEQ ID NO: 6 - DNA, 60 bp, synthetic construct
  misc_feature 1..60: note = Description of Artificial Sequence: Synthetic oligonucleotide
  source 1..60: mol_type = other DNA
cccgtcgctatcaaggaattaagagaagcaacatctgtgggggtccatggctctgaacct

SEQ ID NO: 7 - DNA, 83 bp, synthetic construct
  misc_feature 1..83: note = Description of Artificial Sequence: Synthetic oligonucleotide
  source 1..83: mol_type = other DNA
cccgtcgctatcaaggaattaagagaagcaacatctgtgggggtccatggctctgaacctcaggcccaccttttcttccggtt

SEQ ID NO: 8 - DNA, 67 bp, synthetic construct
  misc_feature 1..67: note = Description of Artificial Sequence: Synthetic probe
  source 1..67: mol_type = other DNA
gactggagttcagacgtgtgctcttccgatctaggttcagagccatggacccccacatttttttttt

SEQ ID NO: 9 - DNA, 24 bp, synthetic construct
  misc_feature 1..24: note = Description of Artificial Sequence: Synthetic primer
  source 1..24: mol_type = other DNA
cccgtcgctatcaaggaattaaga

SEQ ID NO: 10 - DNA, 21 bp, synthetic construct
  misc_feature 1..21: note = Description of Artificial Sequence: Synthetic primer
  source 1..21: mol_type = other DNA
gactggagttcagacgtgtgc

SEQ ID NO: 11 - DNA, 92 bp, synthetic construct
  misc_feature 1..92: note = Description of Artificial Sequence: Synthetic oligonucleotide
  source 1..92: mol_type = other DNA
cccgtcgctatcaaggaattaagagaagcaacatctgtgggggtccatggctctgaacctagatcggaagagcacacgtctgaactccagtc

SEQ ID NO: 12 - DNA, 36 bp, synthetic construct
  misc_feature 1..36: note = Description of Artificial Sequence: Synthetic oligonucleotide
  source 1..36: mol_type = other DNA
tgtgggggtccatggctctgaacctcaggcccacct

SEQ ID NO: 13 - DNA, 24 bp, synthetic construct
  misc_feature 1..24: note = Description of Artificial Sequence: Synthetic primer
  source 1..24: mol_type = other DNA
cccgtcgctatcaaggaattaaga

SEQ ID NO: 14 - DNA, 24 bp, synthetic construct
  misc_feature 1..24: note = Description of Artificial Sequence: Synthetic primer
  source 1..24: mol_type = other DNA
ccacacagcaaagcagaaactcac

SEQ ID NO: 15 - DNA, 21 bp, synthetic construct
  misc_feature 1..21: note = Description of Artificial Sequence: Synthetic primer
  source 1..21: mol_type = other DNA
gactggagttcagacgtgtgc